European Patent Application EP 4 632 071 A1, published October 15, 2025. Title: A microorganism introduced with exogenous soluble pyridine nucleotide transhydrogenase, and method for producing L-tryptophan using the same. Applicant: CJ CheilJedang Corporation. The sequence listing filed with the application follows.

SEQUENCE LISTING (40 sequences)

SEQ ID NO: 1 - protein, 464 aa, Pseudomonas aeruginosa
MAVYNYDVVILGTGPAGEGAAMNASKYGRKLAVVDSRRVVGGNCTHLGTIPSKALRHSVKQIIEFNTNPMFRQIGEPRWFSFPDVLKSADRVISKQVASRTGYYARNRIDMFTGTASFVDERTVEVVTPSGAVERLVADQFVIATGSRPYRPSDINFNHPRVYDSDTILSLSHTPRRLIIYGAGVIGCEYASIFSGLGVLVDLIDTRDQLLSFLDDEISDALSYHLRNNNVLIRHNEEYERVEGLDNGVILHLKSGKKIKADALLWCNGRTGNTDKLGLENVGIKVNSRGQIEVDENYRTSVSNIFAAGDVIGWPSLASAAYDQGRSAAGNIVESDSWRFVNDVPTGIYTIPEISSIGKNESELTAAKIPYEVGKAFFKGMARAQISNEPVGMLKILFHRETLEILGVHCFGDQASEIVHIGQAIMNQPGELNTLKYFVNTTFNYPTMAEAYRVAAFDGLNRLF

SEQ ID NO: 2 - DNA, 1395 bp, Pseudomonas aeruginosa
  source 1..1395: mol_type = genomic DNA
atggctgtctacaactacgacgtggtgattttgggcacgggtccggcgggcgaaggggcggcgatgaacgcctccaagtacggacgcaagctggcggtagtcgacagccgtcgcgtggtcggaggcaactgcacgcacctcggcaccattccttccaaggccctgcgccactcggtgaagcagatcatcgagttcaacaccaacccgatgttccgccagatcggcgagccgcgctggttctccttccccgacgtgctgaagagcgccgaccgggtgatctccaagcaggtcgcttcgcgtaccggctactacgcgcgcaatcgcatcgacatgttcaccggcaccgccagcttcgtcgacgaacgcaccgtcgaagtggtgacgccgagcggcgcggtggagcgcctggtcgccgaccagttcgtgatcgccaccggctcgcgcccgtatcgtccttcggacatcaatttcaaccacccgcgggtctacgacagcgacaccatcctgtccctgagccacaccccgcgccggctgatcatctacggagccggggtgatcggctgcgaatacgcgtcgatcttcagcggcctgggcgtgctggtggacctgatcgatacgcgcgaccagttgctcagcttcctcgatgacgagatttccgatgcgctgagctaccacctgcgcaacaacaacgtgctgatccgccacaacgaggagtacgagcgcgtcgaggggctggacaacggtgtcatcctgcacctgaagtcgggcaagaagatcaaggcggacgcgctgctctggtgcaacggccggaccggcaacaccgacaagctcggcctggagaacgtcggcatcaaggtcaacagccgtggccagatcgaggtggacgagaactaccgcacttcggtgagcaacatcttcgccgccggcgacgtgatcggctggccgagcctggccagcgctgcctacgaccagggccgctcggccgccggcaacatcgtcgagagcgacagctggcgcttcgtcaacgatgtgccgaccggcatctacaccattccggagatcagctcgatcggcaagaacgaaagcgaactgaccgcggcgaagattccctacgaagtgggcaaggcgttcttcaagggcatggcccgggcgcagatttccaacgagccggtgggcatgctgaagatcctgttccatcgcgagaccctggagatcctcggcgtgcactgcttcggcgaccaggcttcggaaatcgtccacatcggtcaggcgatcatgaaccagccgggcgagctgaataccctgaagtacttcgtcaacaccaccttcaactacccgaccatggcggaagcctatcgggtagcggcgttcgacggcctcaaccggcttttttga

SEQ ID NO: 3 - protein, 466 aa, Erwinia amylovora
MQKSYDYDAIVIGSGPGGEGAAMGLVKQGARIAVIERYHNIGGGCTHWGTIPSKALRHAVSRIIEFNQNPLYSDHTRLLRSSFADILKHTENVISQQTHMRQGFYERNHCQIYQGDARFVDANTLEIESHDGSIERLTAEKFVIACGSRPYHPPDVDFSHPRIYDSDSILNLHHEPGHVIIYGAGVIGCEYASIFRGLAVKVDLINTRDRLLAFLDQEMSDSLSYHFWNNGVVIRHNEEFDKVEGVADGVIMHLKSGKKLKADCLLYANGRTGNTDSLFLENVGLEADGRGLLKVNSMYQTAQPHIYAVGDVIGYPSLASAAYDQGRIAAQAMIKGEATAHLIEDIPTGIYTIPEISSVGKTEQQLTAMKVPYEVGRAQFKHLARAQIVGMNVGSLKILFHRETKEILGIHCFGERAAEIIHIGQAIMEQKNGGNTIEYFVNTTFNYPTMAEAYRVAALNGLNRLF

SEQ ID NO: 4 - DNA, 1401 bp, Erwinia amylovora
  source 1..1401: mol_type = genomic DNA
atgcaaaagtcttatgattacgacgccattgtcattggatcaggtcccggcggtgaaggtgccgcaatggggctggtgaaacagggtgcgcgcatcgccgtgattgagcgctatcacaatatcggcggcggttgtacacattgggggaccatcccttcgaaagcgctgcgccacgctgtcagccgtattatcgagttcaaccaaaatcccctctatagcgaccatacacgtcttctgcgttcctctttcgccgacatcctcaagcacaccgaaaatgtgattagccagcaaacccatatgcgccagggcttctatgaacgcaaccactgccagatctatcagggggatgcgcgttttgttgatgccaacaccctcgaaattgaaagccatgacggcagcattgaacggctgacggcggaaaagttcgtcattgcctgtggttctcgtccttatcacccaccggacgtcgatttcagccacccgcgtatctatgacagtgactcgatcctcaatctgcaccatgagccaggccatgtgattatctatggtgccggagtgatcggctgtgaatacgcatctattttccgcgggcttgccgttaaagtcgatttgattaatacccgtgaccgcctgctggcattcctcgaccaggaaatgtcagattctctttcctatcatttctggaataacggggtggtgatccgccataacgaagagttcgacaaggttgaaggagtggctgatggcgtcatcatgcacctgaaatcgggtaaaaagctgaaagctgactgcctgctgtacgccaatggccgtaccggcaataccgattcattgtttctggaaaatgttggactggaagcagacggtcgcggcctgctgaaagtgaacagcatgtaccagacggcacagccgcatatctatgcggtaggtgatgtgattggttacccaagcctggcctcggcagcctacgatcaggggcgtattgccgcacaggcaatgatcaaaggggaagcaaccgcccatctgattgaagatatcccaaccgggatctacaccatcccggaaatcagctccgtcgggaaaaccgagcagcagctgacggcgatgaaagtgccctacgaagtgggccgggcgcagtttaagcaccttgcgcgcgcgcagatcgtcggcatgaacgtcggcagcctgaaaatcctgttccaccgtgaaaccaaagagatccttggcattcactgctttggcgaacgtgccgccgagattattcatatcggtcaggcgatcatggaacagaaaaacggtggcaacacgattgagtacttcgtgaataccacctttaactacccgacaatggcggaagcctaccgggttgcggcgctaaacggcctgaaccggctattttag

SEQ ID NO: 5 - protein, 444 aa, Alteromonas mediterranea
MQLAKAGKKVAVVERYEAVGGGCTHWGTIPSKALRHSVSRLIEYNSSPLFADNHLSKSLTFSDIMRHASGVVKSQTRLRSSFYDRNRVTLFYGEASFVDAHTLEITREDGSKDTVTAAQIAIATGSRPYCPKDIDFNHPRVYNSDTILSLDHDPKSIIIYGAGVIGSEYASIFRGLGVKVDLVNMRDRLLSFLDDEISDALSYHLWNNGVLIRHNETYSSVETLDDSVILNLESGKRMRADCLLFANGRTGNTDTLKLENVGLKADNRGQLRVNENYQTEIDNIYAVGDVIGYPSLASAAYNQGRFAAEAMLGISTHSALVADIPSGIYTIPEISSVGKTEQELTAAKVPYEVGRAQFKHLARAQIASTQTGSLKILFHRETKEILGIHCFGERASEIVHIGQAIMQQKGEGNTIDYFVNTTFNYPTMAEAYRVAAINGLNRIF

SEQ ID NO: 6 - DNA, 1335 bp, Alteromonas mediterranea
  source 1..1335: mol_type = genomic DNA
atgcaacttgccaaggccggtaaaaaagtggctgttgtagagcgctatgaagcggtgggtggaggctgtacgcattggggaaccatcccctcgaaagcgcttcgtcattcagttagccggctcattgagtacaactcatcgcctctgtttgccgataaccatttaagcaagagccttacgttctcagatatcatgcgtcatgccagtggcgttgtgaaaagccaaacacgccttcgctcttccttttacgatagaaaccgggtgacactgttttacggcgaagcaagctttgttgatgcgcatactttagagataacgcgtgaagatggttcaaaagacacggttactgcagcgcaaatagctatcgctactggttcccgtccctactgcccgaaagacatcgattttaatcatccaagggtttataactcagataccattttgtcgttagatcacgaccctaaatccatcataatctacggtgcgggtgttatcggttctgaatatgccagcatttttagagggttaggtgttaaagttgatctggttaacatgcgcgatcgcttactttcatttctagatgatgaaatttccgacgccctgagttaccacttatggaataacggcgttctcattcgccacaacgaaacgtattcatcggtcgaaacgttagatgactctgtgattttaaaccttgaatcaggtaagcgaatgcgagcagactgtttactgtttgctaacgggcgtacgggtaacaccgatacccttaagctggagaatgttggtcttaaagcagacaacagagggcaactgcgcgtaaacgaaaactatcagacagagatagataatatctatgccgtcggtgatgtcattggctaccctagtttagcatcagcggcatataaccaaggccggtttgcagcagaagccatgcttggaataagcactcattcagcgcttgttgccgatatcccttccggtatttacactattccggaaataagctccgtaggcaagacagagcaggagttaacagccgctaaagtgccttatgaagtaggacgagcacagttcaagcatttggctagagcacaaattgcgtccacgcaaaccggtagtcttaagattctctttcatcgtgaaacaaaagaaattttgggcattcactgcttcggagagcgtgcctcagaaattgtgcacatcgggcaagctatcatgcagcaaaaaggtgaaggtaataccattgactacttcgttaataccacatttaactatccgactatggctgaagcctatcgcgttgcagcgataaacggcttgaacaggattttctaa

SEQ ID NO: 7 - protein, 462 aa, Spongiibacter sp. IMCC21906
MAYDYDVVVLGSGPAGESAALNASKHGRTVAVVEAQSLVGGACSHQGTIPSKALRHMVRQAIRFNQTQIFRDLGDPRTLTYPKLLSHAEDVISQQVAMRSRFYYRNNITLIHGQAEFVDAHSIAVLREDGKQSKLTAKQIVIATGSRPYRPADIDFNHPRVYDSDSILKMTNTPRKIIVYGAGVIGCEYASIFSGIGMKVELVNTRDRLLEFLDDEISDALSYHLRYTGVMMRHREEYEKVEADDNGVTLYLKSGKRLHCDALLWCNGRSGNTDNLKLSTIGLEADHRGQLSVNEHYQTAVQDIYAAGDVIGWPSLASAAYDQGRAAAATARGKEHCRFVDDVPTGIYTLPEISSFGLSERELTEEKIPYEVGRAFFKDTARGQISGETVGMLKLLFHVDTLEILGIHCFGAEAAEIIHIGQAIMKQPGDGNTLRYFVNTTFNYPTMAEAYRTAALNGLNRL

SEQ ID NO: 8 - DNA, 1389 bp, Spongiibacter sp. IMCC21906
  source 1..1389: mol_type = genomic DNA
atggcatatgattacgacgttgtggtactgggaagtggtcctgcaggtgaatcggcggccttaaatgccagtaaacatggccgtactgtggcggtggttgaggcgcaatcgctggtcggcggcgcctgttctcatcagggtacgattccctccaaggcacttagacatatggtgcgtcaggctattcgatttaatcaaactcagatttttcgagatttgggtgacccccgaacactgacttaccccaagctgttaagtcatgctgaagatgttatttctcagcaggtggcaatgcgcagccgcttttactaccgcaacaatatcacccttattcacggccaggccgagtttgtcgatgcgcatagcattgcggtattacgtgaggacggcaagcagagcaagctgactgccaagcaaattgtgatcgctactgggtcgaggccttatcgcccagccgatatcgattttaatcacccgcgggtgtatgacagcgacagtattttgaagatgaccaacaccccacgaaaaatcatcgtatacggggccggggtaattggctgtgaatatgcgtcgattttttcgggcattggtatgaaagttgagctggtgaatacccgggatcgcttgttggagtttcttgacgatgaaatttctgacgcccttagttatcacctgcgctataccggtgtgatgatgcggcaccgggaagaatatgagaaggttgaggcagacgataacggcgttaccttgtatctcaaatcgggaaaacgtctgcattgtgacgccttgctttggtgtaatggccgcagtggcaacaccgacaatctcaagttgtcgacgattggccttgaggccgatcatcgcggccagctcagtgtgaatgaacattatcaaaccgccgtacaagacatttacgcggcgggtgacgtgattggttggcccagcctggccagtgcggcttatgaccaaggtagagcggctgcggcgacagcacggggtaaagagcattgccgctttgttgatgatgtgcccaccgggatatacaccttgccagaaatcagttcttttggtttgagtgagcgggagctgactgaagaaaagataccctacgaagtaggccgggcgttttttaaggataccgcccgcgggcaaatcagcggtgaaacggtggggatgttaaagctcttgtttcatgtcgataccttggagattttgggaatccactgttttggggccgaggcggcagaaatcatccatatcggccaggcgattatgaagcagcccggcgacggtaataccctacggtattttgtgaatacgacctttaactatcccaccatggcggaggcttatcgcaccgcggcgcttaatggcttaaatcggttataa

SEQ ID NO: 9 - protein, 471 aa, Amycolatopsis albispora
MSAYDYDLIVIGSGPGGQKAAIAAAKLGKRVAVVDRHDMVGGVCVNTGTIPSKTLREAVHYLTGMSQRELYGASYRVKQDITIADLMARTQHVIGREVEVVRAQLMRNGVHLVSGLGRFTDPHTVAVEGGPRGERTSLTGEYVVIATGTRPARPPEVDFDEARVLDSDEILSLDRIPSSLVVVGAGVIGIEYASMFAALGCRVTVVEQRERMLEFCDPEIVESLKFHLRDLAVTFRFGEKVVDVAVGEHATVTSLASGKRIPAEAVMYSAGRQGMTDALGLEHAGLTADKRGRLAVDDHYRTEVPHIYAVGDVIGFPALAATSMDQGRLAAYHAFGEPANELAALQPIGIYTIPEISYCGATEAELTSSSIPYEIGTARYRELARGQIAGDSYGMLKLLVSTEDRKLLGVHVFGTGATDLVHIGQAVMGCGGTVDYLVDTVFNYPTLSEAYKVAALDATNKIRALARFTTT

SEQ ID NO: 10 - DNA, 1416 bp, Amycolatopsis albispora
  source 1..1416: mol_type = genomic DNA
atgagcgcctatgactacgacctgatcgtgatcggctcgggccccggcgggcagaaggccgccatcgccgcggccaagctcggcaagcgcgtggcggtggtcgaccgccacgacatggtcggcggggtgtgcgtcaacaccggcaccattccgtcgaaaacgctgcgtgaggccgtgcactacctgaccgggatgagccagcgtgagctgtacggggccagctaccgggtcaagcaggacatcaccatcgccgacctgatggcccgcacgcagcacgtgatcgggcgcgaggtcgaggtggtgcgcgcgcagctgatgcgcaacggggtgcacctggtcagcggcctcggccggttcaccgacccgcacaccgtcgcggtcgaaggcggtccgcgtggcgagcggacctcactgaccggtgagtacgtggtgatcgccaccggcacccggccggcgcgcccgccggaggtcgacttcgacgaggcccgcgtgctggactccgacgagatcctgagcctggaccgcatcccgtcttcgctggtcgtggtgggtgccggggtgatcggcatcgagtacgcctcgatgttcgccgcgctgggctgccgggtgaccgtggtcgagcagcgggagcggatgctggagttctgcgacccggagatcgtcgaatcgctgaagttccatctccgggacctggcggtgaccttccggttcggcgagaaggtggtcgacgtggcggtcggcgagcacgccacggtgacgtcgctggccagcgggaagcgcatcccggccgaggcggtgatgtactcggccggtcgccagggcatgaccgacgcgctcggcctggagcacgcgggcctgaccgccgacaagcgcggccgcctcgccgtcgacgaccactaccgcaccgaggtcccgcacatctacgccgtcggtgacgtgatcggcttccccgcgctcgccgcgacttcgatggaccagggcaggctggccgcgtaccacgccttcggcgaaccggcgaacgagctggccgcgctgcagccgatcggcatctacaccattccggagatctcctactgcggcgcgaccgaggccgagctgacgtcttcttcgatcccgtacgagatcggtaccgcccggtaccgcgaactggcccgaggccaaatcgccggcgactcgtatggcatgctcaagctgctggtgtccacagaggaccggaaactgctgggcgtgcacgtcttcggcaccggggccaccgacctggtccacatcggacaagccgtaatgggctgcggcggcacggtcgactacctggtggacaccgtgttcaactacccgacgctgtcggaggcgtacaaggtcgccgcactggacgccaccaacaagatccgcgcactggcccgcttcaccacaacctga

SEQ ID NO: 11 - protein, 464 aa, Azotobacter vinelandii
MAVYNYDVVVIGTGPAGEGAAMNAVKAGRKVAVVDDRPQVGGNCTHLGTIPSKALRHSVRQIMQYNNNPLFRQIGEPRWFSFADVLKSAEQVIAKQVSSRTGYYARNRIDTFFGTASFCDEHTIEVVHLNGMVETLVAKQFVIATGSRPYRPADVDFTHPRIYDSDTILSLGHTPRRLIIYGAGVIGCEYASIFSGLGVLVDLIDNRDQLLSFLDDEISDSLSYHLRNNNVLIRHNEEYERVEGLDNGVILHLKSGKKIKADAFLWSNGRTGNTDKLGLENIGLKANGRGQIQVDEHYRTEVSNIYAAGDVIGWPSLASAAYDQGRSAAGSITENDSWRFVDDVPTGIYTIPEISSVGKTERELTQAKVPYEVGKAFFKGMARAQIAVEKAGMLKILFHRETLEILGVHCFGYQASEIVHIGQAIMNQKGEANTLKYFINTTFNYPTMAEAYRVAAYDGLNRLF

SEQ ID NO: 12 - DNA, 1395 bp, Azotobacter vinelandii
  source 1..1395: mol_type = genomic DNA
atggctgtatataactacgatgtggtggtaatcggcacaggccctgctggcgaaggggcagcgatgaatgccgtgaaggccgggcgcaaggtagcggtcgtggatgatcgcccccaggtcggcggcaactgcacccacctcggaaccattccctccaaggcgctgcgccactcggtgcggcagatcatgcagtacaacaacaatccgctgttccgccagatcggcgagccgcgctggttttccttcgccgatgtcctgaagagcgccgagcaggtcatcgccaagcaggtttcctcgcggaccggctactatgcgcgcaaccgtatcgataccttcttcgggaccgcgagcttctgcgacgagcacaccatcgaggtcgtccacctcaacggtatggtggaaacgctggtggccaagcagttcgtcatcgccaccgggtcgcgtccctaccgcccggccgatgtcgatttcacccatccgcgcatctacgacagcgacaccatcctcagcctcggccacacgccgcgccggttgatcatctacggagcgggggtgatcggctgcgaatatgcctccatcttcagtgggctgggcgtgctggtcgacctcatcgacaaccgcgaccaactgctcagtttcctcgacgacgaaatctccgactcgctcagctaccacctgcgcaacaacaacgtgctgatccgccacaacgaggaatacgagcgtgtcgaaggcctggacaacggggtgatcctgcacctcaagtccggcaagaagatcaaggccgacgccttcctgtggagcaacggccgtaccggcaataccgacaagctgggcctggagaacatcggtctcaaggccaatggtcgcggacagatccaggtcgacgagcactaccgtaccgaagtcagcaacatctatgccgctggtgacgtgatcggctggccgagcctggccagcgccgcctatgaccagggtcgttcggccgcgggcagtatcaccgagaacgatagctggcgtttcgtcgacgacgtgccgaccggcatctacaccattccggagatcagttcggtcggcaagaccgagcgcgaactgacccaggcgaaggttccctacgaggtcggcaaggccttcttcaagggcatggcccgggcacagatcgccgtcgagaaggccggcatgctgaagatcctctttcaccgcgagacgctggaaatcctcggcgtgcactgcttcggctatcaggcttcggaaatcgtccatatcggccaggcgatcatgaaccagaagggcgaggcgaataccctcaagtatttcatcaacaccaccttcaactacccgaccatggccgaggcctaccgggtggcggcctacgacggtctcaatcggcttttttga

SEQ ID NO: 13 - DNA, 32 bp, synthetic construct
  source 1..32: mol_type = other DNA
caggaattcgatctgaatttcacgcgcaacgg

SEQ ID NO: 14 - DNA, 36 bp, synthetic construct
  source 1..36: mol_type = other DNA
gttgtagacagccatggtagggcttacctgttctta

SEQ ID NO: 15 - DNA, 36 bp, synthetic construct
  source 1..36: mol_type = other DNA
caggtaagccctaccatggctgtctacaactacgac

SEQ ID NO: 16 - DNA, 35 bp, synthetic construct
  source 1..35: mol_type = other DNA
catttcgataaagtttcaaaaaagccggttgaggc

SEQ ID NO: 17 - DNA, 37 bp, synthetic construct
  source 1..37: mol_type = other DNA
aaccggcttttttgaaactttatcgaaatggccatcc

SEQ ID NO: 18 - DNA, 40 bp, synthetic construct
  source 1..40: mol_type = other DNA
gctaggtcgactagcgtgatggaatgctgctggtggatca

SEQ ID NO: 19 - DNA, 36 bp, synthetic construct
  source 1..36: mol_type = other DNA
ataagacttttgcatggtagggcttacctgttctta

SEQ ID NO: 20 - DNA, 40 bp, synthetic construct
  source 1..40: mol_type = other DNA
caggtaagccctaccatgcaaaagtcttatgattacgacg

SEQ ID NO: 21 - DNA, 36 bp, synthetic construct
  source 1..36: mol_type = other DNA
catttcgataaagttctaaaatagccggttcaggcc

SEQ ID NO: 22 - DNA, 37 bp, synthetic construct
  source 1..37: mol_type = other DNA
aaccggctattttagaactttatcgaaatggccatcc

SEQ ID NO: 23 - DNA, 36 bp, synthetic construct
  source 1..36: mol_type = other DNA
cttggcaagttgcatggtagggcttacctgttctta

SEQ ID NO: 24 - DNA, 35 bp, synthetic construct
  source 1..35: mol_type = other DNA
caggtaagccctaccatgcaacttgccaaggccgg

SEQ ID NO: 25 - DNA, 40 bp, synthetic construct
  source 1..40: mol_type = other DNA
catttcgataaagttttagaaaatcctgttcaagccgttt

SEQ ID NO: 26 - DNA, 37 bp, synthetic construct
  source 1..37: mol_type = other DNA
aacaggattttctaaaactttatcgaaatggccatcc

SEQ ID NO: 27 - DNA, 36 bp, synthetic construct
  source 1..36: mol_type = other DNA
gtaatcatatgccatggtagggcttacctgttctta

SEQ ID NO: 28 - DNA, 39 bp, synthetic construct
  source 1..39: mol_type = other DNA
caggtaagccctaccatggcatatgattacgacgttgtg

SEQ ID NO: 29 - DNA, 40 bp, synthetic construct
  source 1..40: mol_type = other DNA
catttcgataaagttttataaccgatttaagccattaagc

SEQ ID NO: 30 - DNA, 37 bp, synthetic construct
  source 1..37: mol_type = other DNA
ttaaatcggttataaaactttatcgaaatggccatcc

SEQ ID NO: 31 - DNA, 36 bp, synthetic construct
  source 1..36: mol_type = other DNA
gtcataggcgctcatggtagggcttacctgttctta

SEQ ID NO: 32 - DNA, 36 bp, synthetic construct
  source 1..36: mol_type = other DNA
caggtaagccctaccatgagcgcctatgactacgac

SEQ ID NO: 33 - DNA, 35 bp, synthetic construct
  source 1..35: mol_type = other DNA
catttcgataaagtttcaggttgtggtgaagcggg

SEQ ID NO: 34 - DNA, 37 bp, synthetic construct
  source 1..37: mol_type = other DNA
ttcaccacaacctgaaactttatcgaaatggccatcc

SEQ ID NO: 35 - DNA, 36 bp, synthetic construct
  source 1..36: mol_type = other DNA
gttatatacagccatggtagggcttacctgttctta

SEQ ID NO: 36 - DNA, 40 bp, synthetic construct
  source 1..40: mol_type = other DNA
caggtaagccctaccatggctgtatataactacgatgtgg

SEQ ID NO: 37 - DNA, 37 bp, synthetic construct
  source 1..37: mol_type = other DNA
catttcgataaagtttcaaaaaagccgattgagaccg

SEQ ID NO: 38 - DNA, 37 bp, synthetic construct
  source 1..37: mol_type = other DNA
aatcggcttttttgaaactttatcgaaatggccatcc

SEQ ID NO: 39 - DNA, 18 bp, synthetic construct
  source 1..18: mol_type = other DNA
cagtaaacgcacgcggca

SEQ ID NO: 40 - DNA, 18 bp, synthetic construct
  source 1..18: mol_type = other DNA
gtgatgttgctggagcgg